European Patent Application EP 4 144 760 A1, published March 8, 2023. Title: ANTIGEN BINDING CONSTRUCTS TARGETING HER2 AND USES THEREOF. Applicant: CHIA TAI TIANQING PHARMACEUTICAL GROUP CO., LTD. Application WO PCT/CN2021/090794, filed April 29, 2021. The sequence listing filed with the application follows.

SEQUENCE LISTING (55 sequences)

SEQ ID NO: 1 - protein, 475 aa, synthetic construct
  REGION 1..475: note = Amino acid sequence of anti-Her2-scFv-Fc
EVQLVESGGGLVQPGGSLRLSCAASGFNIKDTYIHWVRQAPGKGLEWVARIYPTNGYTRYADSVKGRFTISADTSKNTAYLQMNSLRAEDTAVYYCSRWGGDGFYAMDYWGQGTLVTVSSGGGGSGGGGSGGGGSDIQMTQSPSSLSASVGDRVTITCRASQDVNTAVAWYQQKPGKAPKLLIYSASFLYSGVPSRFSGSRSGTDFTLTISSLQPEDFATYYCQQHYTTPPTFGQGTKVEIKGEPKSSDKTHTCPPCPAPELLGGPSVFLFPPKPKDTLMISRTPEVTCVVVDVSHEDPEVKFNWYVDGVEVHNAKTKPREEQYNSTYRVVSVLTVLHQDWLNGKEYKCKVSNKALPAPIEKTISKAKGQPREPQVYTLPPSREEMTKNQVSLTCLVKGFYPSDIAVEWESNGQPENNYKTTPPVLDSDGSFFLYSKLTVDKSRWQQGNVFSCSVMHEALHNHYTQKSLSLSPGK

SEQ ID NO: 2 - DNA, 1425 bp, synthetic construct
  misc_feature 1..1425: note = Nucleotide sequence of anti-Her2-scFv-Fc
  source 1..1425: mol_type = other DNA
gaggtgcagctggtggagtctggaggaggactggtgcagccaggaggcagcctgcggctgtcttgtgccgcttccggcttcaacatcaaggacacctacatccattgggtgaggcaggctccaggcaagggactggagtgggtggctcggatctatcctaccaatggctacacaagatatgccgactccgtgaagggccggtttaccatcagcgccgatacctctaagaacacagcttacctgcagatgaattccctgagggccgaggacacagccgtgtactattgcagcagatggggaggcgacggcttctacgctatggattattggggccagggcaccctggtgacagtgtccagcggcggcggcggctctggaggaggaggatccggaggaggaggaagcgatatccagatgacccagtccccttcttccctgtctgcctccgtgggcgacagagtgaccatcacatgtcgcgctagccaggatgtgaacacagccgtggcttggtaccagcagaagccaggcaaggcccccaagctgctgatctactccgcctccttcctgtattccggagtgccaagcaggttttccggaagccggtctggaaccgacttcaccctgacaatcagctctctgcagcctgaggattttgccacatactattgccagcagcactataccacaccccctaccttcggccagggcacaaaggtggagatcaagggcgagccaaagtccagcgacaagacccatacatgcccaccatgtcctgctccagagctgctgggcggcccttccgtgttcctgtttcctccaaagccaaaggataccctgatgatctctagaacccctgaggtgacatgcgtggtggtggacgtgtcccacgaggatccagaggtgaagtttaactggtacgtggacggcgtggaggtgcataatgccaagaccaagccaagagaggagcagtacaattctacctatcgcgtggtgtccgtgctgacagtgctgcaccaggattggctgaacggcaaggagtataagtgcaaggtgagcaataaggccctgcccgctcccatcgagaagaccatctctaaggctaagggccagcccagagagcctcaggtgtacacactgccccctagccgcgaggagatgaccaagaaccaggtgtctctgacatgtctggtgaagggcttttatccatctgacatcgccgtggagtgggagtccaatggccagcccgagaacaattacaagaccacaccacccgtgctggactctgatggctccttctttctgtattccaagctgaccgtggataagagccgctggcagcagggcaacgtgttctcctgcagcgtgatgcatgaggctctgcacaatcattacacacagaagtctctgtccctgagccctggcaag

SEQ ID NO: 3 - protein, 475 aa, synthetic construct
  REGION 1..475: note = Amino acid sequence of anti-Her2-scFv-VL-F53Y-Fc
EVQLVESGGGLVQPGGSLRLSCAASGFNIKDTYIHWVRQAPGKGLEWVARIYPTNGYTRYADSVKGRFTISADTSKNTAYLQMNSLRAEDTAVYYCSRWGGDGFYAMDYWGQGTLVTVSSGGGGSGGGGSGGGGSDIQMTQSPSSLSASVGDRVTITCRASQDVNTAVAWYQQKPGKAPKLLIYSASYLYSGVPSRFSGSRSGTDFTLTISSLQPEDFATYYCQQHYTTPPTFGQGTKVEIKGEPKSSDKTHTCPPCPAPELLGGPSVFLFPPKPKDTLMISRTPEVTCVVVDVSHEDPEVKFNWYVDGVEVHNAKTKPREEQYNSTYRVVSVLTVLHQDWLNGKEYKCKVSNKALPAPIEKTISKAKGQPREPQVYTLPPSREEMTKNQVSLTCLVKGFYPSDIAVEWESNGQPENNYKTTPPVLDSDGSFFLYSKLTVDKSRWQQGNVFSCSVMHEALHNHYTQKSLSLSPGK

SEQ ID NO: 4 - DNA, 1425 bp, synthetic construct
  misc_feature 1..1425: note = Nucleotide sequence of anti-Her2-scFv-VL-F53Y-Fc
  source 1..1425: mol_type = other DNA
gaggtgcagctggtggagtctggaggaggactggtgcagccaggaggcagcctgcggctgtcttgtgccgcttccggcttcaacatcaaggacacctacatccattgggtgaggcaggctccaggcaagggactggagtgggtggctcggatctatcctaccaatggctacacaagatatgccgactccgtgaagggccggtttaccatcagcgccgatacctctaagaacacagcttacctgcagatgaattccctgagggccgaggacacagccgtgtactattgcagcagatggggaggcgacggcttctacgctatggattattggggccagggcaccctggtgacagtgtccagcggcggcggcggctctggaggaggaggatccggaggaggaggaagcgatatccagatgacccagtccccttcttccctgtctgcctccgtgggcgacagagtgaccatcacatgtcgcgctagccaggatgtgaacacagccgtggcttggtaccagcagaagccaggcaaggcccccaagctgctgatctactccgcctcctacctgtattccggagtgccaagcaggttttccggaagccggtctggaaccgacttcaccctgacaatcagctctctgcagcctgaggattttgccacatactattgccagcagcactataccacaccccctaccttcggccagggcacaaaggtggagatcaagggcgagccaaagtccagcgacaagacccatacatgcccaccatgtcctgctccagagctgctgggcggcccttccgtgttcctgtttcctccaaagccaaaggataccctgatgatctctagaacccctgaggtgacatgcgtggtggtggacgtgtcccacgaggatccagaggtgaagtttaactggtacgtggacggcgtggaggtgcataatgccaagaccaagccaagagaggagcagtacaattctacctatcgcgtggtgtccgtgctgacagtgctgcaccaggattggctgaacggcaaggagtataagtgcaaggtgagcaataaggccctgcccgctcccatcgagaagaccatctctaaggctaagggccagcccagagagcctcaggtgtacacactgccccctagccgcgaggagatgaccaagaaccaggtgtctctgacatgtctggtgaagggcttttatccatctgacatcgccgtggagtgggagtccaatggccagcccgagaacaattacaagaccacaccacccgtgctggactctgatggctccttctttctgtattccaagctgaccgtggataagagccgctggcagcagggcaacgtgttctcctgcagcgtgatgcatgaggctctgcacaatcattacacacagaagtctctgtccctgagccctggcaag

SEQ ID NO: 5 - protein, 475 aa, synthetic construct
  REGION 1..475: note = Amino acid sequence of anti-Her2-scFv-VL-F53A-Fc
EVQLVESGGGLVQPGGSLRLSCAASGFNIKDTYIHWVRQAPGKGLEWVARIYPTNGYTRYADSVKGRFTISADTSKNTAYLQMNSLRAEDTAVYYCSRWGGDGFYAMDYWGQGTLVTVSSGGGGSGGGGSGGGGSDIQMTQSPSSLSASVGDRVTITCRASQDVNTAVAWYQQKPGKAPKLLIYSASALYSGVPSRFSGSRSGTDFTLTISSLQPEDFATYYCQQHYTTPPTFGQGTKVEIKGEPKSSDKTHTCPPCPAPELLGGPSVFLFPPKPKDTLMISRTPEVTCVVVDVSHEDPEVKFNWYVDGVEVHNAKTKPREEQYNSTYRVVSVLTVLHQDWLNGKEYKCKVSNKALPAPIEKTISKAKGQPREPQVYTLPPSREEMTKNQVSLTCLVKGFYPSDIAVEWESNGQPENNYKTTPPVLDSDGSFFLYSKLTVDKSRWQQGNVFSCSVMHEALHNHYTQKSLSLSPGK

SEQ ID NO: 6 - DNA, 1425 bp, synthetic construct
  misc_feature 1..1425: note = Nucleotide sequence of anti-Her2-scFv-VL-F53A-Fc
  source 1..1425: mol_type = other DNA
gaggtgcagctggtggagtctggaggaggactggtgcagccaggaggcagcctgcggctgtcttgtgccgcttccggcttcaacatcaaggacacctacatccattgggtgaggcaggctccaggcaagggactggagtgggtggctcggatctatcctaccaatggctacacaagatatgccgactccgtgaagggccggtttaccatcagcgccgatacctctaagaacacagcttacctgcagatgaattccctgagggccgaggacacagccgtgtactattgcagcagatggggaggcgacggcttctacgctatggattattggggccagggcaccctggtgacagtgtccagcggcggcggcggctctggaggaggaggatccggaggaggaggaagcgatatccagatgacccagtccccttcttccctgtctgcctccgtgggcgacagagtgaccatcacatgtcgcgctagccaggatgtgaacacagccgtggcttggtaccagcagaagccaggcaaggcccccaagctgctgatctactccgcctccgccctgtattccggagtgccaagcaggttttccggaagccggtctggaaccgacttcaccctgacaatcagctctctgcagcctgaggattttgccacatactattgccagcagcactataccacaccccctaccttcggccagggcacaaaggtggagatcaagggcgagccaaagtccagcgacaagacccatacatgcccaccatgtcctgctccagagctgctgggcggcccttccgtgttcctgtttcctccaaagccaaaggataccctgatgatctctagaacccctgaggtgacatgcgtggtggtggacgtgtcccacgaggatccagaggtgaagtttaactggtacgtggacggcgtggaggtgcataatgccaagaccaagccaagagaggagcagtacaattctacctatcgcgtggtgtccgtgctgacagtgctgcaccaggattggctgaacggcaaggagtataagtgcaaggtgagcaataaggccctgcccgctcccatcgagaagaccatctctaaggctaagggccagcccagagagcctcaggtgtacacactgccccctagccgcgaggagatgaccaagaaccaggtgtctctgacatgtctggtgaagggcttttatccatctgacatcgccgtggagtgggagtccaatggccagcccgagaacaattacaagaccacaccacccgtgctggactctgatggctccttctttctgtattccaagctgaccgtggataagagccgctggcagcagggcaacgtgttctcctgcagcgtgatgcatgaggctctgcacaatcattacacacagaagtctctgtccctgagccctggcaag

SEQ ID NO: 7 - protein, 475 aa, synthetic construct
  REGION 1..475: note = Amino acid sequence of anti-Her2-scFv-VL-F53R-Fc
EVQLVESGGGLVQPGGSLRLSCAASGFNIKDTYIHWVRQAPGKGLEWVARIYPTNGYTRYADSVKGRFTISADTSKNTAYLQMNSLRAEDTAVYYCSRWGGDGFYAMDYWGQGTLVTVSSGGGGSGGGGSGGGGSDIQMTQSPSSLSASVGDRVTITCRASQDVNTAVAWYQQKPGKAPKLLIYSASRLYSGVPSRFSGSRSGTDFTLTISSLQPEDFATYYCQQHYTTPPTFGQGTKVEIKGEPKSSDKTHTCPPCPAPELLGGPSVFLFPPKPKDTLMISRTPEVTCVVVDVSHEDPEVKFNWYVDGVEVHNAKTKPREEQYNSTYRVVSVLTVLHQDWLNGKEYKCKVSNKALPAPIEKTISKAKGQPREPQVYTLPPSREEMTKNQVSLTCLVKGFYPSDIAVEWESNGQPENNYKTTPPVLDSDGSFFLYSKLTVDKSRWQQGNVFSCSVMHEALHNHYTQKSLSLSPGK

SEQ ID NO: 8 - DNA, 1425 bp, synthetic construct
  misc_feature 1..1425: note = Nucleotide sequence of anti-Her2-scFv-VL-F53R-Fc
  source 1..1425: mol_type = other DNA
gaggtgcagctggtggagtctggaggaggactggtgcagccaggaggcagcctgcggctgtcttgtgccgcttccggcttcaacatcaaggacacctacatccattgggtgaggcaggctccaggcaagggactggagtgggtggctcggatctatcctaccaatggctacacaagatatgccgactccgtgaagggccggtttaccatcagcgccgatacctctaagaacacagcttacctgcagatgaattccctgagggccgaggacacagccgtgtactattgcagcagatggggaggcgacggcttctacgctatggattattggggccagggcaccctggtgacagtgtccagcggcggcggcggctctggaggaggaggatccggaggaggaggaagcgatatccagatgacccagtccccttcttccctgtctgcctccgtgggcgacagagtgaccatcacatgtcgcgctagccaggatgtgaacacagccgtggcttggtaccagcagaagccaggcaaggcccccaagctgctgatctactccgcctccaggctgtattccggagtgccaagcaggttttccggaagccggtctggaaccgacttcaccctgacaatcagctctctgcagcctgaggattttgccacatactattgccagcagcactataccacaccccctaccttcggccagggcacaaaggtggagatcaagggcgagccaaagtccagcgacaagacccatacatgcccaccatgtcctgctccagagctgctgggcggcccttccgtgttcctgtttcctccaaagccaaaggataccctgatgatctctagaacccctgaggtgacatgcgtggtggtggacgtgtcccacgaggatccagaggtgaagtttaactggtacgtggacggcgtggaggtgcataatgccaagaccaagccaagagaggagcagtacaattctacctatcgcgtggtgtccgtgctgacagtgctgcaccaggattggctgaacggcaaggagtataagtgcaaggtgagcaataaggccctgcccgctcccatcgagaagaccatctctaaggctaagggccagcccagagagcctcaggtgtacacactgccccctagccgcgaggagatgaccaagaaccaggtgtctctgacatgtctggtgaagggcttttatccatctgacatcgccgtggagtgggagtccaatggccagcccgagaacaattacaagaccacaccacccgtgctggactctgatggctccttctttctgtattccaagctgaccgtggataagagccgctggcagcagggcaacgtgttctcctgcagcgtgatgcatgaggctctgcacaatcattacacacagaagtctctgtccctgagccctggcaag

SEQ ID NO: 9 - protein, 475 aa, synthetic construct
  REGION 1..475: note = Amino acid sequence of anti-Her2-scFv-VH-K30E-Fc
EVQLVESGGGLVQPGGSLRLSCAASGFNIEDTYIHWVRQAPGKGLEWVARIYPTNGYTRYADSVKGRFTISADTSKNTAYLQMNSLRAEDTAVYYCSRWGGDGFYAMDYWGQGTLVTVSSGGGGSGGGGSGGGGSDIQMTQSPSSLSASVGDRVTITCRASQDVNTAVAWYQQKPGKAPKLLIYSASFLYSGVPSRFSGSRSGTDFTLTISSLQPEDFATYYCQQHYTTPPTFGQGTKVEIKGEPKSSDKTHTCPPCPAPELLGGPSVFLFPPKPKDTLMISRTPEVTCVVVDVSHEDPEVKFNWYVDGVEVHNAKTKPREEQYNSTYRVVSVLTVLHQDWLNGKEYKCKVSNKALPAPIEKTISKAKGQPREPQVYTLPPSREEMTKNQVSLTCLVKGFYPSDIAVEWESNGQPENNYKTTPPVLDSDGSFFLYSKLTVDKSRWQQGNVFSCSVMHEALHNHYTQKSLSLSPGK

SEQ ID NO: 10 - DNA, 1425 bp, synthetic construct
  misc_feature 1..1425: note = Nucleotide sequence of anti-Her2-scFv-VH-K30E-Fc
  source 1..1425: mol_type = other DNA
gaggtgcagctggtggagtctggaggaggactggtgcagccaggaggcagcctgcggctgtcttgtgccgcttccggcttcaacatcgaggacacctacatccattgggtgaggcaggctccaggcaagggactggagtgggtggctcggatctatcctaccaatggctacacaagatatgccgactccgtgaagggccggtttaccatcagcgccgatacctctaagaacacagcttacctgcagatgaattccctgagggccgaggacacagccgtgtactattgcagcagatggggaggcgacggcttctacgctatggattattggggccagggcaccctggtgacagtgtccagcggcggcggcggctctggaggaggaggatccggaggaggaggaagcgatatccagatgacccagtccccttcttccctgtctgcctccgtgggcgacagagtgaccatcacatgtcgcgctagccaggatgtgaacacagccgtggcttggtaccagcagaagccaggcaaggcccccaagctgctgatctactccgcctccttcctgtattccggagtgccaagcaggttttccggaagccggtctggaaccgacttcaccctgacaatcagctctctgcagcctgaggattttgccacatactattgccagcagcactataccacaccccctaccttcggccagggcacaaaggtggagatcaagggcgagccaaagtccagcgacaagacccatacatgcccaccatgtcctgctccagagctgctgggcggcccttccgtgttcctgtttcctccaaagccaaaggataccctgatgatctctagaacccctgaggtgacatgcgtggtggtggacgtgtcccacgaggatccagaggtgaagtttaactggtacgtggacggcgtggaggtgcataatgccaagaccaagccaagagaggagcagtacaattctacctatcgcgtggtgtccgtgctgacagtgctgcaccaggattggctgaacggcaaggagtataagtgcaaggtgagcaataaggccctgcccgctcccatcgagaagaccatctctaaggctaagggccagcccagagagcctcaggtgtacacactgccccctagccgcgaggagatgaccaagaaccaggtgtctctgacatgtctggtgaagggcttttatccatctgacatcgccgtggagtgggagtccaatggccagcccgagaacaattacaagaccacaccacccgtgctggactctgatggctccttctttctgtattccaagctgaccgtggataagagccgctggcagcagggcaacgtgttctcctgcagcgtgatgcatgaggctctgcacaatcattacacacagaagtctctgtccctgagccctggcaag

SEQ ID NO: 11 - protein, 480 aa, synthetic construct
  REGION 1..480: note = Amino acid sequence of anti-Her2-scFv-VH-K30E-VL-F53Y-Fc
EVQLVESGGGLVQPGGSLRLSCAASGFNIEDTYIHWVRQAPGKGLEWVARIYPTNGYTRYADSVKGRFTISADTSKNTAYLQMNSLRAEDTAVYYCSRWGGDGFYAMDYWGQGTLVTVSSGGGGSGGGGSGGGGSGGGGSDIQMTQSPSSLSASVGDRVTITCRASQDVNTAVAWYQQKPGKAPKLLIYSASYLYSGVPSRFSGSRSGTDFTLTISSLQPEDFATYYCQQHYTTPPTFGQGTKVEIKGEPKSSDKTHTCPPCPAPELLGGPSVFLFPPKPKDTLMISRTPEVTCVVVDVSHEDPEVKFNWYVDGVEVHNAKTKPREEQYNSTYRVVSVLTVLHQDWLNGKEYKCKVSNKALPAPIEKTISKAKGQPREPQVYTLPPCREEMTKNQVSLWCLVKGFYPSDIAVEWESNGQPENNYKTTPPVLDSDGSFFLYSKLTVDKSRWQQGNVFSCSVMHEALHNHYTQKSLSLSPGK

SEQ ID NO: 12 - DNA, 1443 bp, synthetic construct
  misc_feature 1..1443: note = Nucleotide sequence of anti-Her2-scFv-VH-K30E-VL-F53Y-Fc
  source 1..1443: mol_type = other DNA
gaggtgcaactggtggaatccggcgggggactggtccaacctggagggagcctgcggctgtcttgcgccgcctctggcttcaacatcgaggatacctacatccactgggtgcggcaggcccctggcaagggcctggaatgggtcgctagaatctaccctaccaacggctacaccagatacgccgactctgtaaagggcagattcaccatctctgccgatacatctaagaacaccgcctacctgcagatgaactccctgagagccgaggacaccgccgtgtactactgctcccggtggggcggtgacggcttttacgccatggactactggggacaaggcacacttgttacggtgtcctctggaggcggcggctccggcggcggcggctctggcggaggcggctctggcggcggcggatctgatatccagatgacccagtctcctagctccctctccgcctccgtgggcgacagagtgacaatcacctgcagagcttctcaggacgtgaacaccgctgtggcctggtaccagcagaagcctggcaaggcccctaagctgctgatctactctgcttcctacctgtactccggcgtgcccagccggttctccggctctcggtccggcaccgacttcactctgaccatctccagcctgcagcctgaagatttcgccacctactactgccagcagcactacaccacccctcccaccttcggccagggcaccaaagtggagatcaagggcgagcccaagtcctccgataaaacccacacctgtcctccttgccctgcccctgaactactgggcggcccttctgtgttcctgttccctcctaagcccaaggacaccctgatgatctctagaacccctgaagtgacctgcgtggtggtggatgtgtctcacgaggaccctgaggtcaagttcaactggtacgtggacggcgtggaagtgcataacgccaagaccaagcctagagaagagcagtacaactccacctacagagtggtctccgtgctgaccgtgctgcaccaggactggctgaacggcaaagagtacaagtgcaaggtgtccaacaaggctctgcctgctcctatcgagaagacaatctccaaggccaaaggccagcctcgggagcctcaggtgtacaccctgcctccttgtagagaggaaatgaccaagaaccaggtgtctctgtggtgcctggtgaagggcttctacccatccgacatcgccgtcgagtgggagtccaacggacagcccgagaacaactacaagactaccccacctgtgctggactccgatggctccttcttcctgtactccaagctgaccgtggacaagtccagatggcagcagggcaacgtgttctcctgctccgtgatgcacgaggccctgcacaaccactacacccagaaatccctgtctctgtcccctggcaagtga

SEQ ID NO: 13 - protein, 449 aa, synthetic construct
  REGION 1..449: note = Amino acid sequence of anti-Her2-domain2-HC-Fc
EVQLVESGGGLVQPGGSLRLSCAASGFTFTDYTMDWVRQAPGKGLEWVADVNPNSGGSIYNQRFKGRFTLSVDRSKNTLYLQMNSLRAEDTAVYYCARNLGPSFYFDYWGQGTLVTVSSASTKGPSVFPLAPSSKSTSGGTAALGCLVKDYFPEPVTVSWNSGALTSGVHTFPAVLQSSGLYSLSSVVTVPSSSLGTQTYICNVNHKPSNTKVDKKVEPKSCDKTHTCPPCPAPELLGGPSVFLFPPKPKDTLMISRTPEVTCVVVDVSHEDPEVKFNWYVDGVEVHNAKTKPREEQYNSTYRVVSVLTVLHQDWLNGKEYKCKVSNKALPAPIEKTISKAKGQPREPQVCTLPPSREEMTKNQVSLSCAVKGFYPSDIAVEWESNGQPENNYKTTPPVLDSDGSFFLVSKLTVDKSRWQQGNVFSCSVMHEALHNRFTQKSLSLSPGK

SEQ ID NO: 14 - DNA, 1350 bp, synthetic construct
  misc_feature 1..1350: note = Nucleotide sequence of anti-Her2-domain2-HC-Fc
  source 1..1350: mol_type = other DNA
gaagtgcagctggttgaatctggcggcggattggttcagcctggcggatctctgagactgtcttgtgccgcctctggcttcaccttcaccgactacaccatggactgggtccgacaggctcctggcaaaggactggaatgggtcgccgacgtgaaccctaattccggcggctccatctacaaccagcggttcaagggcagattcaccctgtccgtggaccggtctaagaacaccctgtacctgcagatgaactccctgagagccgaggacaccgccgtgtactactgcgccagaaacctgggaccttccttctacttcgactactggggccagggcaccctggtcacagtttcttccgcttccaccaagggacccagcgtgttccctctggctccttccagcaagtctacctctggcggaacagctgctctgggctgcctggtcaaggactactttcctgagcctgtgaccgtgtcctggaactctggcgctctgacatctggcgtgcacacctttccagctgtgctgcagtcctccggcctgtactctctgtcctctgtcgtgaccgtgccttccagctctctgggaacccagacctacatctgcaatgtgaaccacaagccttccaacaccaaggtggacaagaaggtggaacccaagtcctgcgacaagacccacacctgtcctccatgtcctgctccagaactgctcggcggaccttccgtgttcctgtttcctccaaagcctaaggataccctgatgatctctcggacccctgaagtgacctgcgtggtggtggatgtgtctcacgaggatcccgaagtgaagttcaattggtacgtggacggcgtggaagtgcacaacgccaagaccaagcctagagaggaacagtacaactccacctacagagtggtgtccgtgctgaccgtgctgcaccaggattggctgaacggcaaagagtacaagtgcaaggtgtccaacaaggccctgcctgctcctatcgaaaagaccatctccaaggccaagggccagcctcgggaacctcaagtctgtaccctgcctcctagccgggaagagatgaccaagaaccaggtgtccctgtcctgtgccgtgaagggcttctacccttccgatatcgccgtggaatgggagagcaatggccagcctgagaacaactacaagacaacccctcctgtgctggactccgacggctcattcttcctggtgtccaagctgacagtggacaagtccagatggcagcagggcaacgtgttctcctgctccgtgatgcacgaggccctgcacaacaggttcacccagaagtccctgtctctgagccccggcaaatga

SEQ ID NO: 15 - protein, 214 aa, synthetic construct
  REGION 1..214: note = Amino acid sequence of anti-Her2-domain2-LC
DIQMTQSPSSLSASVGDRVTITCKASQDVSIGVAWYQQKPGKAPKLLIYSASYRYTGVPSRFSGSGSGTDFTLTISSLQPEDFATYYCQQYYIYPYTFGQGTKVEIKRTVAAPSVFIFPPSDEQLKSGTASVVCLLNNFYPREAKVQWKVDNALQSGNSQESVTEQDSKDSTYSLSSTLTLSKADYEKHKVYACEVTHQGLSSPVTKSFNRGEC

SEQ ID NO: 16 - DNA, 645 bp, synthetic construct
  misc_feature 1..645: note = Nucleotide sequence of anti-Her2-domain2-LC
  source 1..645: mol_type = other DNA
gatatccagatgacccagtctccttccagcctgtctgcctctgtgggcgacagagtgaccatcacatgcaaggcctctcaggacgtgtccatcggcgtggcatggtatcagcagaagcctggcaaggcccctaagctgctgatctactccgcctcctacagatacacaggcgtgccctccagattctccggctctggctctggcacagactttaccctgacaatctccagcctgcagcctgaggacttcgccacctactactgccagcagtactacatctacccctacaccttcggccagggcaccaaggtggaaatcaagagaaccgtggccgctccttccgtgttcatcttcccaccttccgacgagcagctgaagtctggcaccgcttctgtcgtgtgcctgctgaacaacttctaccctcgggaagccaaggtgcagtggaaggtggacaatgccctgcagtccggcaactcccaagagtctgtgaccgagcaggactccaaggacagcacctatagcctgtcctccacactgaccctgtccaaggccgactacgagaagcacaaggtgtacgcctgcgaagtgacccatcagggcctgtctagtcccgtgaccaagtctttcaaccggggcgagtgttga

SEQ ID NO: 17 - protein, 481 aa, synthetic construct
  REGION 1..481: note = Amino acid sequence of anti-Her2-scFv-VL-VH-Fc
DIQMTQSPSSLSASVGDRVTITCRASQDVNTAVAWYQQKPGKAPKLLIYSASFLYSGVPSRFSGSRSGTDFTLTISSLQPEDFATYYCQQHYTTPPTFGQGTKVEIKGGSGGGSGGGSGGGSGGGSGEVQLVESGGGLVQPGGSLRLSCAASGFNIKDTYIHWVRQAPGKGLEWVARIYPTNGYTRYADSVKGRFTISADTSKNTAYLQMNSLRAEDTAVYYCSRWGGDGFYAMDYWGQGTLVTVSSAAEPKSSDKTHTCPPCPAPELLGGPSVFLFPPKPKDTLMISRTPEVTCVVVDVSHEDPEVKFNWYVDGVEVHNAKTKPREEQYNSTYRVVSVLTVLHQDWLNGKEYKCKVSNKALPAPIEKTISKAKGQPREPQVYTLPPSRDELTKNQVSLICLVKGFYPSDIAVEWESNGQPENRYMTWPPVLDSDGSFFLYSKLTVDKSRWQQGNVFSCSVMHEALHNHYTQKSLSLSPGK

SEQ ID NO: 18 - DNA, 1443 bp, synthetic construct
  misc_feature 1..1443: note = Nucleotide sequence of anti-Her2-scFv-VL-VH-Fc
  source 1..1443: mol_type = other DNA
gatatccagatgacccagtccccttcctcactgtctgcctccgtgggagacagagtgacaatcacctgcagagcttcccaggatgtgaacaccgcagtggcctggtaccagcagaagcctggcaaggctcctaagctgctgatctactctgcttccttcctgtactccggcgtcccttctcggttctctggctcccggtctggcaccgactttaccctgaccatctccagcctgcagcctgaagacttcgccacctactactgccagcagcactacaccactccacccaccttcggtcagggcaccaaggtcgagatcaagggcggctccggcgggggctccggcggcggctctggcggcggaagcggaggcggaagtggcgaagtgcaactggtcgagtctggaggcggcctggttcagcctggcggaagcctacggctgtcttgcgccgcctctggctttaacatcaaggacacctacatccactgggtgcggcaggctcccggcaagggcctggaatgggtggccagaatctaccctaccaatggctacaccagatacgccgattctgtgaaaggtagattcacaatctccgccgacacctccaagaataccgcctacctgcagatgaactccctgagagccgaggatacagctgtctactactgttccagatggggcggcgatggcttctacgccatggactactggggccagggcacactggtgaccgtgtcctccgctgctgagcctaagtcctccgacaaaacccacacctgtcccccttgtcctgctccagaactcctgggcggcccttccgtgtttctgttccccccgaagcctaaagataccctgatgatctctcgcaccccagaagtgacatgcgtggtagtcgacgtgtctcatgaggaccctgaggtgaagttcaactggtatgtggacggcgtggaagtgcacaacgccaagaccaagcctagagaagagcagtacaactctacctaccgggtggtgtctgtgctgacagtgctgcaccaggactggctgaacggcaaagagtacaagtgcaaggtgtccaacaaggccctgcctgctcccatcgagaagaccatttctaaggccaagggacagcccagagaacctcaagtgtataccctgcctcctagccgggacgagctgaccaagaaccaggtgtccctgatctgcctggtgaagggcttctaccccagcgacatcgccgtggagtgggagtccaacggccaacctgagaaccggtacatgacctggcctcctgtgctggactccgacggcagcttcttcctgtactctaagctgaccgtggacaagagtagatggcagcaaggcaacgtgttctcctgctcggtgatgcacgaggctctgcataaccactacacccagaaatccctgtctttgagccctggcaag

SEQ ID NO: 19 - protein, 448 aa, synthetic construct
  REGION 1..448: note = Amino acid sequence of anti-Her2-domain2-HC-Fc-2
EVQLVESGGGLVQPGGSLRLSCAASGFTFTDYTMDWVRQAPGKGLEWVADVNPNSGGSIYNQRFKGRFTLSVDRSKNTLYLQMNSLRAEDTAVYYCARNLGPSFYFDYWGQGTLVTVSSASTKGPSVFPLAPSSKSTSGGTAALGCLVKDYFPEPVTVSWNSGALTSGVHTFPAVLQSSGLYSLSSVVTVPSSSLGTQTYICNVNHKPSNTKVDKKVEPKSCDKTHTCPPCPAPELLGGPSVFLFPPKPKDTLMISRTPEVTCVVVDVSHEDPEVKFNWYVDGVEVHNAKTKPREEQYNSTYRVVSVLTVLHQDWLNGKEYKCKVSNKALPAPIEKTISKAKGQPREPQVYVYPPSRDELTKNQVSLTCLVKGFYPSDIAVEWESNGQPENNYKTTPPVLDSDGSFALVSKLTVDKSRWQQGNVFSCSVMHEALHNRFTQKSLSLSPG

SEQ ID NO: 20 - DNA, 1344 bp, synthetic construct
  misc_feature 1..1344: note = Nucleotide sequence of anti-Her2-domain2-HC-Fc-2
  source 1..1344: mol_type = other DNA
gaggtgcagctggtcgagtctggaggaggtctggtgcagcctggaggctctctgcggctgtcctgtgccgcttctggcttcaccttcaccgactacaccatggactgggtgcggcaggcccctggcaaggggctggaatgggtggccgacgtgaatcctaactctggcggctccatctacaaccagcggttcaagggcagattcacactgtccgtggacagatccaagaacaccctgtacctgcagatgaacagcctgagagccgaggacaccgctgtgtactactgcgcccggaacctgggacccagcttctacttcgactactggggccaaggcaccctggtcaccgtgtccagcgccagcaccaaaggccctagtgtctttcctctggctcccagctctaagtccacctccggcggcaccgctgctctgggctgtctggtgaaggactatttccctgagcctgtgaccgtctcttggaactccggcgctctgacctctggcgtgcatacctttcccgccgtgctgcagtccagcggcctgtactctttgtcttctgtcgtgacagtgccttcttcctctctcggcacacagacctacatctgcaacgtgaaccacaagccatctaacaccaaagtggacaagaaggtggaacccaagagctgcgacaaaacccacacctgtccaccttgtcctgcccctgagctgctgggcggaccttccgtgttcctgttcccccctaagcctaaggatacactgatgatctccagaacccccgaggtgacctgcgtggtggtggatgtttcccatgaagatcctgaagtgaagttcaactggtacgtggacggcgtggaagtgcacaacgccaagaccaagcctagagaggaacagtacaactctacctacagagtggtttctgtgctcactgtgctgcaccaggattggctgaacggcaaagagtacaagtgcaaggtgtccaacaaggccctgcctgctcctatcgagaagaccatcagcaaggctaagggccagcctcgcgaacctcaggtgtacgtgtatcctccttcccgggacgagctgaccaagaaccaagtgtctctgacctgcctggtgaaaggcttctacccctccgacatcgccgtggaatgggagtccaatggccagcccgagaacaactacaagaccacccctccagtgctggactccgatggctccttcgccctggtgtccaagctgacagtagacaagtctagatggcagcagggcaacgtgttctcctgctccgtgatgcacgaggccctgcacaatagattcacacagaagtccctgtctctgtcccctggc

SEQ ID NO: 21 - protein, 480 aa, synthetic construct
  REGION 1..480: note = Amino acid sequence of b-anti-Her2-scFv-VH-K30E-Fc
EVQLVESGGGLVQPGGSLRLSCAASGFNIEDTYIHWVRQAPGKGLEWVARIYPTNGYTRYADSVKGRFTISADTSKNTAYLQMNSLRAEDTAVYYCSRWGGDGFYAMDYWGQGTLVTVSSGGGGSGGGGSGGGGSGGGGSDIQMTQSPSSLSASVGDRVTITCRASQDVNTAVAWYQQKPGKAPKLLIYSASFLYSGVPSRFSGSRSGTDFTLTISSLQPEDFATYYCQQHYTTPPTFGQGTKVEIKGEPKSSDKTHTCPPCPAPELLGGPSVFLFPPKPKDTLMISRTPEVTCVVVDVSHEDPEVKFNWYVDGVEVHNAKTKPREEQYNSTYRVVSVLTVLHQDWLNGKEYKCKVSNKALPAPIEKTISKAKGQPREPQVYTLPPCREEMTKNQVSLWCLVKGFYPSDIAVEWESNGQPENNYKTTPPVLDSDGSFFLYSKLTVDKSRWQQGNVFSCSVMHEALHNHYTQKSLSLSPGK

SEQ ID NO: 22 - DNA, 1443 bp, synthetic construct
  misc_feature 1..1443: note = Nucleotide sequence of b-anti-Her2-scFv-VH-K30E-Fc
  source 1..1443: mol_type = other DNA
gaggtgcaactggtggaatccggcgggggactggtccaacctggagggagcctgcggctgtcttgcgccgcctctggcttcaacatcgaggatacctacatccactgggtgcggcaggcccctggcaagggcctggaatgggtcgctagaatctaccctaccaacggctacaccagatacgccgactctgtaaagggcagattcaccatctctgccgatacatctaagaacaccgcctacctgcagatgaactccctgagagccgaggacaccgccgtgtactactgctcccggtggggcggtgacggcttttacgccatggactactggggacaaggcacacttgttacggtgtcctctggaggcggcggctccggcggcggcggctctggcggaggcggctctggcggcggcggatctgatatccagatgacccagtctcctagctccctctccgcctccgtgggcgacagagtgacaatcacctgcagagcttctcaggacgtgaacaccgctgtggcctggtaccagcagaagcctggcaaggcccctaagctgctgatctactctgcttccttcctgtactccggcgtgcccagccggttctccggctctcggtccggcaccgacttcactctgaccatctccagcctgcagcctgaagatttcgccacctactactgccagcagcactacaccacccctcccaccttcggccagggcaccaaagtggagatcaagggcgagcccaagtcctccgataaaacccacacctgtcctccttgccctgcccctgaactactgggcggcccttctgtgttcctgttccctcctaagcccaaggacaccctgatgatctctagaacccctgaagtgacctgcgtggtggtggatgtgtctcacgaggaccctgaggtcaagttcaactggtacgtggacggcgtggaagtgcataacgccaagaccaagcctagagaagagcagtacaactccacctacagagtggtctccgtgctgaccgtgctgcaccaggactggctgaacggcaaagagtacaagtgcaaggtgtccaacaaggctctgcctgctcctatcgagaagacaatctccaaggccaaaggccagcctcgggagcctcaggtgtacaccctgcctccttgtagagaggaaatgaccaagaaccaggtgtctctgtggtgcctggtgaagggcttctacccatccgacatcgccgtcgagtgggagtccaacggacagcccgagaacaactacaagactaccccacctgtgctggactccgatggctccttcttcctgtactccaagctgaccgtggacaagtccagatggcagcagggcaacgtgttctcctgctccgtgatgcacgaggccctgcacaaccactacacccagaaatccctgtctctgtcccctggcaagtga

SEQ ID NO: 23 - protein, 480 aa, synthetic construct
  REGION 1..480: note = Amino acid sequence of b-anti-Her2-scFv-VL-F53Y-Fc
EVQLVESGGGLVQPGGSLRLSCAASGFNIKDTYIHWVRQAPGKGLEWVARIYPTNGYTRYADSVKGRFTISADTSKNTAYLQMNSLRAEDTAVYYCSRWGGDGFYAMDYWGQGTLVTVSSGGGGSGGGGSGGGGSGGGGSDIQMTQSPSSLSASVGDRVTITCRASQDVNTAVAWYQQKPGKAPKLLIYSASYLYSGVPSRFSGSRSGTDFTLTISSLQPEDFATYYCQQHYTTPPTFGQGTKVEIKGEPKSSDKTHTCPPCPAPELLGGPSVFLFPPKPKDTLMISRTPEVTCVVVDVSHEDPEVKFNWYVDGVEVHNAKTKPREEQYNSTYRVVSVLTVLHQDWLNGKEYKCKVSNKALPAPIEKTISKAKGQPREPQVYTLPPCREEMTKNQVSLWCLVKGFYPSDIAVEWESNGQPENNYKTTPPVLDSDGSFFLYSKLTVDKSRWQQGNVFSCSVMHEALHNHYTQKSLSLSPGK

SEQ ID NO: 24 - DNA, 1443 bp, synthetic construct
  misc_feature 1..1443: note = Nucleotide sequence of b-anti-Her2-scFv-VL-F53Y-Fc
  source 1..1443: mol_type = other DNA
gaggtgcaactggtggaatccggcgggggactggtccaacctggagggagcctgcggctgtcttgcgccgcctctggcttcaacatcaaggatacctacatccactgggtgcggcaggcccctggcaagggcctggaatgggtcgctagaatctaccctaccaacggctacaccagatacgccgactctgtaaagggcagattcaccatctctgccgatacatctaagaacaccgcctacctgcagatgaactccctgagagccgaggacaccgccgtgtactactgctcccggtggggcggtgacggcttttacgccatggactactggggacaaggcacacttgttacggtgtcctctggaggcggcggctccggcggcggcggctctggcggaggcggctctggcggcggcggatctgatatccagatgacccagtctcctagctccctctccgcctccgtgggcgacagagtgacaatcacctgcagagcttctcaggacgtgaacaccgctgtggcctggtaccagcagaagcctggcaaggcccctaagctgctgatctactctgcttcctacctgtactccggcgtgcccagccggttctccggctctcggtccggcaccgacttcactctgaccatctccagcctgcagcctgaagatttcgccacctactactgccagcagcactacaccacccctcccaccttcggccagggcaccaaagtggagatcaagggcgagcccaagtcctccgataaaacccacacctgtcctccttgccctgcccctgaactactgggcggcccttctgtgttcctgttccctcctaagcccaaggacaccctgatgatctctagaacccctgaagtgacctgcgtggtggtggatgtgtctcacgaggaccctgaggtcaagttcaactggtacgtggacggcgtggaagtgcataacgccaagaccaagcctagagaagagcagtacaactccacctacagagtggtctccgtgctgaccgtgctgcaccaggactggctgaacggcaaagagtacaagtgcaaggtgtccaacaaggctctgcctgctcctatcgagaagacaatctccaaggccaaaggccagcctcgggagcctcaggtgtacaccctgcctccttgtagagaggaaatgaccaagaaccaggtgtctctgtggtgcctggtgaagggcttctacccatccgacatcgccgtcgagtgggagtccaacggacagcccgagaacaactacaagactaccccacctgtgctggactccgatggctccttcttcctgtactccaagctgaccgtggacaagtccagatggcagcagggcaacgtgttctcctgctccgtgatgcacgaggccctgcacaaccactacacccagaaatccctgtctctgtcccctggcaagtga

SEQ ID NO: 25 - protein, 480 aa, synthetic construct
  REGION 1..480: note = Amino acid sequence of anti-Her2-scFv-VH-VL-Fc
EVQLVESGGGLVQPGGSLRLSCAASGFNIKDTYIHWVRQAPGKGLEWVARIYPTNGYTRYADSVKGRFTISADTSKNTAYLQMNSLRAEDTAVYYCSRWGGDGFYAMDYWGQGTLVTVSSGGGGSGGGGSGGGGSGGGGSDIQMTQSPSSLSASVGDRVTITCRASQDVNTAVAWYQQKPGKAPKLLIYSASFLYSGVPSRFSGSRSGTDFTLTISSLQPEDFATYYCQQHYTTPPTFGQGTKVEIKGEPKSSDKTHTCPPCPAPELLGGPSVFLFPPKPKDTLMISRTPEVTCVVVDVSHEDPEVKFNWYVDGVEVHNAKTKPREEQYNSTYRVVSVLTVLHQDWLNGKEYKCKVSNKALPAPIEKTISKAKGQPREPQVYTLPPCREEMTKNQVSLWCLVKGFYPSDIAVEWESNGQPENNYKTTPPVLDSDGSFFLYSKLTVDKSRWQQGNVFSCSVMHEALHNHYTQKSLSLSPGK

SEQ ID NO: 26 - DNA, 1440 bp, synthetic construct
  misc_feature 1..1440: note = Nucleotide sequence of anti-Her2-scFv-VH-VL-Fc
  source 1..1440: mol_type = other DNA
gaggtgcaactggtggaatccggcgggggactggtccaacctggagggagcctgcggctgtcttgcgccgcctctggcttcaacatcaaggatacctacatccactgggtgcggcaggcccctggcaagggcctggaatgggtcgctagaatctaccctaccaacggctacaccagatacgccgactctgtaaagggcagattcaccatctctgccgatacatctaagaacaccgcctacctgcagatgaactccctgagagccgaggacaccgccgtgtactactgctcccggtggggcggtgacggcttttacgccatggactactggggacaaggcacacttgttacggtgtcctctggaggcggcggctccggcggcggcggctctggcggaggcggctctggcggcggcggatctgatatccagatgacccagtctcctagctccctctccgcctccgtgggcgacagagtgacaatcacctgcagagcttctcaggacgtgaacaccgctgtggcctggtaccagcagaagcctggcaaggcccctaagctgctgatctactctgcttccttcctgtactccggcgtgcccagccggttctccggctctcggtccggcaccgacttcactctgaccatctccagcctgcagcctgaagatttcgccacctactactgccagcagcactacaccacccctcccaccttcggccagggcaccaaagtggagatcaagggcgagcccaagtcctccgataaaacccacacctgtcctccttgccctgcccctgaactactgggcggcccttctgtgttcctgttccctcctaagcccaaggacaccctgatgatctctagaacccctgaagtgacctgcgtggtggtggatgtgtctcacgaggaccctgaggtcaagttcaactggtacgtggacggcgtggaagtgcataacgccaagaccaagcctagagaagagcagtacaactccacctacagagtggtctccgtgctgaccgtgctgcaccaggactggctgaacggcaaagagtacaagtgcaaggtgtccaacaaggctctgcctgctcctatcgagaagacaatctccaaggccaaaggccagcctcgggagcctcaggtgtacaccctgcctccttgtagagaggaaatgaccaagaaccaggtgtctctgtggtgcctggtgaagggcttctacccatccgacatcgccgtcgagtgggagtccaacggacagcccgagaacaactacaagactaccccacctgtgctggactccgatggctccttcttcctgtactccaagctgaccgtggacaagtccagatggcagcagggcaacgtgttctcctgctccgtgatgcacgaggccctgcacaaccactacacccagaaatccctgtctctgtcccctggcaag

SEQ ID NO: 27 - protein, 10 aa, synthetic construct
  MUTAGEN 5: note = X is K or E
  REGION 1..10: note = Heavy chain CDR1 of a first antigen-binding fragment
GFNIXDTYIH

SEQ ID NO: 28 - protein, 17 aa, Mus musculus
  REGION 1..17: note = Heavy chain CDR2 of a first antigen-binding fragment
RIYPTNGYTRYADSVKG

SEQ ID NO: 29 - protein, 12 aa, Mus musculus
  REGION 1..12: note = Heavy chain CDR3 of a first antigen-binding fragment
WGGDGFYAMDYW

SEQ ID NO: 30 - protein, 13 aa, Mus musculus
  REGION 1..13: note = Light chain CDR1 of a first antigen-binding fragment
CRASQDVNTAVAW

SEQ ID NO: 31 - protein, 7 aa, synthetic construct
  REGION 1..7: note = Light chain CDR2 of a first antigen-binding fragment
SASYLYS

SEQ ID NO: 32 - protein, 9 aa, Mus musculus
  REGION 1..9: note = Light chain CDR3 of a first antigen-binding fragment
QQHYTTPPT

SEQ ID NO: 33 - protein, 7 aa, Mus musculus
  REGION 1..7: note = Light chain CDR2 of a first antigen-binding fragment
SASFLYS

SEQ ID NO: 34 - protein, 7 aa, synthetic construct
  MUTAGEN 4: note = X is F or Y
  REGION 1..7: note = Light chain CDR2 of a first antigen-binding fragment
SASXLYS

SEQ ID NO: 35 - protein, 120 aa, synthetic construct
  REGION 1..120: note = Amino acid sequence of heavy chain variable region of a first antigen-binding fragment
EVQLVESGGGLVQPGGSLRLSCAASGFNIEDTYIHWVRQAPGKGLEWVARIYPTNGYTRYADSVKGRFTISADTSKNTAYLQMNSLRAEDTAVYYCSRWGGDGFYAMDYWGQGTLVTVSS

SEQ ID NO: 36 - protein, 107 aa, synthetic construct
  REGION 1..107: note = Amino acid sequence of light chain variable region of a first antigen-binding fragment
DIQMTQSPSSLSASVGDRVTITCRASQDVNTAVAWYQQKPGKAPKLLIYSASYLYSGVPSRFSGSRSGTDFTLTISSLQPEDFATYYCQQHYTTPPTFGQGTKVEIK

SEQ ID NO: 37 - protein, 119 aa, synthetic construct [sequence omitted]

SEQ ID NO: 38 - protein, 107 aa, synthetic construct [sequence omitted]

SEQ ID NO: 39 - protein, 107 aa, synthetic construct [sequence omitted]

SEQ ID NO: 40 - protein, 120 aa, synthetic construct [sequence omitted]

SEQ ID NO: 41 - protein, 120 aa, synthetic construct
  MUTAGEN 30: note = X is K or E
  REGION 1..120: note = Amino acid sequence of heavy chain variable region of a first antigen-binding fragment
EVQLVESGGGLVQPGGSLRLSCAASGFNIXDTYIHWVRQAPGKGLEWVARIYPTNGYTRYADSVKGRFTISADTSKNTAYLQMNSLRAEDTAVYYCSRWGGDGFYAMDYWGQGTLVTVSS

SEQ ID NO: 42 - protein, 107 aa, synthetic construct
  MUTAGEN 53: note = X is F or Y
  REGION 1..107: note = Amino acid sequence of light chain variable region of a first antigen-binding fragment
DIQMTQSPSSLSASVGDRVTITCRASQDVNTAVAWYQQKPGKAPKLLIYSASXLYSGVPSRFSGSRSGTDFTLTISSLQPEDFATYYCQQHYTTPPTFGQGTKVEIK

SEQ ID NO: 43 - protein, 10 aa, synthetic construct
  REGION 1..10: note = Heavy chain CDR1 of a first antigen-binding fragment
GFNIEDTYIH

SEQ ID NO: 44 - protein, 10 aa, Mus musculus
GFNIKDTYIH

SEQ ID NO: 45 - protein, 10 aa, Mus musculus
GFTFTDYTMD

SEQ ID NO: 46 - protein, 17 aa, Mus musculus
DVNPNSGGSIYNQRFKG

SEQ ID NO: 47 - protein, 10 aa, Mus musculus
NLGPSFYFDY

SEQ ID NO: 48 - protein, 11 aa, Mus musculus
KASQDVSIGVA

SEQ ID NO: 49 - protein, 7 aa, Mus musculus
SASYRYT

SEQ ID NO: 50 - protein, 9 aa, Mus musculus
QQYYIYPYT

SEQ ID NO: 51 - protein, 475 aa, synthetic construct
  REGION 1..475: note = Amino acid sequence of a bivalent monospecific antibody
EVQLVESGGGLVQPGGSLRLSCAASGFNIEDTYIHWVRQAPGKGLEWVARIYPTNGYTRYADSVKGRFTISADTSKNTAYLQMNSLRAEDTAVYYCSRWGGDGFYAMDYWGQGTLVTVSSGGGGSGGGGSGGGGSDIQMTQSPSSLSASVGDRVTITCRASQDVNTAVAWYQQKPGKAPKLLIYSASYLYSGVPSRFSGSRSGTDFTLTISSLQPEDFATYYCQQHYTTPPTFGQGTKVEIKGEPKSSDKTHTCPPCPAPELLGGPSVFLFPPKPKDTLMISRTPEVTCVVVDVSHEDPEVKFNWYVDGVEVHNAKTKPREEQYNSTYRVVSVLTVLHQDWLNGKEYKCKVSNKALPAPIEKTISKAKGQPREPQVYTLPPSREEMTKNQVSLTCLVKGFYPSDIAVEWESNGQPENNYKTTPPVLDSDGSFFLYSKLTVDKSRWQQGNVFSCSVMHEALHNHYTQKSLSLSPGK

SEQ ID NO: 52 - protein, 14 aa, synthetic construct
  REGION 1..14: note = Amino acid sequence of linker peptide
GGSGGSGGSGGSGG

SEQ ID NO: 53 - protein, 15 aa, synthetic construct
  REGION 1..15: note = Amino acid sequence of linker peptide
GGGGSGGGGSGGGGS

SEQ ID NO: 54 - protein, 20 aa, synthetic construct
  REGION 1..20: note = Amino acid sequence of linker peptide
GGGGSGGGGSGGGGSGGGGS

SEQ ID NO: 55 - protein, 7 aa, synthetic construct
  REGION 1..7: note = Amino acid sequence of linker peptide
GGGPGKR